European Patent Application EP 4 725 968 A1, published April 15, 2026. Title: ANTI-GPC3 ANTIBODY OR ANTIGEN-BINDING FRAGMENT AND USE THEREOF. Applicant: SALUBRIS (CHENGDU) BIOTECH CO., LTD. Application CN, filed June 13, 2024. The sequence listing filed with the application follows.

SEQUENCE LISTING (58 sequences)

SEQ ID NO: 1 - protein, 121 aa, synthetic construct
QVQLLESGGGLVQPGGSLRVSCAASGFTFNSYAMSWVRQAPGKGLEWVASIKSSGDRVQYADSVKGRFTISRDNSKNTVYLEMNSLRAEDTAIYYCAKPQWSSPQRTFEVWGQGTPVTVSS

SEQ ID NO: 2 - protein, 121 aa, synthetic construct
EVQLLESGGGLVQPGGSLRLSCAASGFTFNSYAMSWVRQAPGKGLEWVASIKSSGDRVQYADSVKGRFTISRDNSKNTVYLQMNSLRAEDTAIYYCAKPQWSSPQRTFEVWGQGTMVTVSS

SEQ ID NO: 3 - protein, 107 aa, synthetic construct
DIQLTQSPSSLSASVGDRVTITCRASQSISSYLNWYQQKPGKAPKLLIYAASSLQSGVPSRFSGSGSGTDFTLTISSLQPEDFATYYCQQSYSTPWTFGQGTKVEIK

SEQ ID NO: 4 - protein, 330 aa, synthetic construct
ASTKGPSVFPLAPSSKSTSGGTAALGCLVKDYFPEPVTVSWNSGALTSGVHTFPAVLQSSGLYSLSSVVTVPSSSLGTQTYICNVNHKPSNTKVDKRVEPKSCDKTHTCPPCPAPELLGGPSVFLFPPKPKDTLMISRTPEVTCVVVDVSHEDPEVKFNWYVDGVEVHNAKTKPREEQYNSTYRVVSVLTVLHQDWLNGKEYKCKVSNKALPAPIEKTISKAKGQPREPQVYTLPPSRDELTKNQVSLTCLVKGFYPSDIAVEWESNGQPENNYKTTPPVLDSDGSFFLYSKLTVDKSRWQQGNVFSCSVMHEALHNHYTQKSLSLSPGK

SEQ ID NO: 5 - protein, 107 aa, synthetic construct [sequence omitted]

SEQ ID NO: 6 - protein, 121 aa, synthetic construct
EVQLLESGGGLVQPGGSLRLSCAASGFTFNSYAMSWVRQAPGKGLEWVASIKSSGDRVQYADSVKGRFTISRDNSKNTVYLEMNSLRAEDTAIYYCAKPQWSSPQRTFEVWGQGTPVTVSS

SEQ ID NO: 7 - protein, 121 aa, synthetic construct
QVQLLESGGGLVQPGGSLRVSCAASGFTFNSYAMSWVRQAPGKGLEWVASIKSSGDRVQYADSVKGRFTISRDNSKNTVYLQMNSLRAEDTAIYYCAKPQWSSPQRTFEVWGQGTPVTVSS

SEQ ID NO: 8 - protein, 121 aa, synthetic construct
QVQLLESGGGLVQPGGSLRVSCAASGFTFNSYAMSWVRQAPGKGLEWVASIKSSGDRVQYADSVKGRFTISRDNSKNTVYLEMNSLRAEDTAIYYCAKPQWSSPQRTFEVWGQGTMVTVSS

SEQ ID NO: 9 - protein, 121 aa, synthetic construct
EVQLLESGGGLVQPGGSLRLSCAASGFTFNSYAMSWVRQAPGKGLEWVASIKSSGDRVQYADSVKGRFTISRDNSKNTVYLQMNSLRAEDTAIYYCAKPQWSSPQRTFEVWGQGTPVTVSS

SEQ ID NO: 10 - protein, 214 aa, synthetic construct
DIQLTQSPSSLSASVGDRVTITCRASQSISSYLNWYQQKPGKAPKLLIYAASSLQSGVPSRFSGSGSGTDFTLTISSLQPEDFATYYCQQSYSTPWTFGQGTKVEIKRTVAAPSVFIFPPSDEQLKSGTASVVCLLNNFYPREAKVQWKVDNALQSGNSQESVTEQDSKDSTYSLSSTLTLSKADYEKHKVYACEVTHQGLSSPVTKSFNRGEC

SEQ ID NO: 11 - protein, 451 aa, synthetic construct
QVQLLESGGGLVQPGGSLRVSCAASGFTFNSYAMSWVRQAPGKGLEWVASIKSSGDRVQYADSVKGRFTISRDNSKNTVYLEMNSLRAEDTAIYYCAKPQWSSPQRTFEVWGQGTPVTVSSASTKGPSVFPLAPSSKSTSGGTAALGCLVKDYFPEPVTVSWNSGALTSGVHTFPAVLQSSGLYSLSSVVTVPSSSLGTQTYICNVNHKPSNTKVDKRVEPKSCDKTHTCPPCPAPELLGGPSVFLFPPKPKDTLMISRTPEVTCVVVDVSHEDPEVKFNWYVDGVEVHNAKTKPREEQYNSTYRVVSVLTVLHQDWLNGKEYKCKVSNKALPAPIEKTISKAKGQPREPQVYTLPPSRDELTKNQVSLTCLVKGFYPSDIAVEWESNGQPENNYKTTPPVLDSDGSFFLYSKLTVDKSRWQQGNVFSCSVMHEALHNHYTQKSLSLSPGK

SEQ ID NO: 12 - protein, 451 aa, synthetic construct
QVQLLESGGGLVQPGGSLRVSCAASGFTFNSYAMSWVRQAPGKGLEWVASIKSSGDRVQYADSVKGRFTISRDNSKNTVYLEMNSLRAEDTAIYYCAKPQWSSPQRTFEVWGQGTPVTVSSASTKGPSVFPLAPSSKSTSGGTAALGCLVKDYFPEPVTVSWNSGALTSGVHTFPAVLQSSGLYSLSSVVTVPSSSLGTQTYICNVNHKPSNTKVDKRVEPKSCDKTHTCPPCPAPEAAGGPCVFLFPPKPKDTLMISRTPEVTCVVVDVSHEDPEVKFNWYVDGVEVHNAKTKPREEQYNSTYRVVSVLTVLHQDWLNGKEYKCKVSNKALGAPIEKTISKAKGQPREPQVYTLPPSRDELTKNQVSLTCLVKGFYPSDIAVEWESNGQPENNYKTTPPVLDSDGSFFLYSKLTVDKSRWQQGNVFSCSVMHEALHNHYTQKSLSLSPGK

SEQ ID NO: 13 - protein, 451 aa, synthetic construct
QVQLLESGGGLVQPGGSLRVSCAASGFTFNSYAMSWVRQAPGKGLEWVASIKSSGDRVQYADSVKGRFTISRDNSKNTVYLEMNSLRAEDTAIYYCAKPQWSSPQRTFEVWGQGTPVTVSSASTKGPSVFPLAPSSKSTSGGTAALGCLVKDYFPEPVTVSWNSGALTSGVHTFPAVLQSSGLYSLSSVVTVPSSSLGTQTYICNVNHKPSNTKVDKRVEPKSCDKTHTCPPCPAPEAAGGPCVFLFPPKPKDTLMISRTPEVTCVVVDVSHEDPEVKFNWYVDGVEVHNAKTKPREEQYNSTYRVVSVLTVLHQDWLNGKEYKCKVSNKALGAPIEKTISKAKGQPREPQVYTLPPSRDELTKNQVSLTCLVKGFYPSDIAVEWESNGQPENNYKTTPPVLDSDGSFFLYSKLTVDKSRWQQGNVFSCSVLHEALHSHYTQKSLSLSPGK

SEQ ID NO: 14 - protein, 451 aa, synthetic construct
EVQLLESGGGLVQPGGSLRLSCAASGFTFNSYAMSWVRQAPGKGLEWVASIKSSGDRVQYADSVKGRFTISRDNSKNTVYLEMNSLRAEDTAIYYCAKPQWSSPQRTFEVWGQGTPVTVSSASTKGPSVFPLAPSSKSTSGGTAALGCLVKDYFPEPVTVSWNSGALTSGVHTFPAVLQSSGLYSLSSVVTVPSSSLGTQTYICNVNHKPSNTKVDKRVEPKSCDKTHTCPPCPAPELLGGPSVFLFPPKPKDTLMISRTPEVTCVVVDVSHEDPEVKFNWYVDGVEVHNAKTKPREEQYNSTYRVVSVLTVLHQDWLNGKEYKCKVSNKALPAPIEKTISKAKGQPREPQVYTLPPSRDELTKNQVSLTCLVKGFYPSDIAVEWESNGQPENNYKTTPPVLDSDGSFFLYSKLTVDKSRWQQGNVFSCSVMHEALHNHYTQKSLSLSPGK

SEQ ID NO: 15 - protein, 451 aa, synthetic construct
QVQLLESGGGLVQPGGSLRVSCAASGFTFNSYAMSWVRQAPGKGLEWVASIKSSGDRVQYADSVKGRFTISRDNSKNTVYLQMNSLRAEDTAIYYCAKPQWSSPQRTFEVWGQGTPVTVSSASTKGPSVFPLAPSSKSTSGGTAALGCLVKDYFPEPVTVSWNSGALTSGVHTFPAVLQSSGLYSLSSVVTVPSSSLGTQTYICNVNHKPSNTKVDKRVEPKSCDKTHTCPPCPAPELLGGPSVFLFPPKPKDTLMISRTPEVTCVVVDVSHEDPEVKFNWYVDGVEVHNAKTKPREEQYNSTYRVVSVLTVLHQDWLNGKEYKCKVSNKALPAPIEKTISKAKGQPREPQVYTLPPSRDELTKNQVSLTCLVKGFYPSDIAVEWESNGQPENNYKTTPPVLDSDGSFFLYSKLTVDKSRWQQGNVFSCSVMHEALHNHYTQKSLSLSPGK

SEQ ID NO: 16 - protein, 451 aa, synthetic construct
QVQLLESGGGLVQPGGSLRVSCAASGFTFNSYAMSWVRQAPGKGLEWVASIKSSGDRVQYADSVKGRFTISRDNSKNTVYLEMNSLRAEDTAIYYCAKPQWSSPQRTFEVWGQGTMVTVSSASTKGPSVFPLAPSSKSTSGGTAALGCLVKDYFPEPVTVSWNSGALTSGVHTFPAVLQSSGLYSLSSVVTVPSSSLGTQTYICNVNHKPSNTKVDKRVEPKSCDKTHTCPPCPAPELLGGPSVFLFPPKPKDTLMISRTPEVTCVVVDVSHEDPEVKFNWYVDGVEVHNAKTKPREEQYNSTYRVVSVLTVLHQDWLNGKEYKCKVSNKALPAPIEKTISKAKGQPREPQVYTLPPSRDELTKNQVSLTCLVKGFYPSDIAVEWESNGQPENNYKTTPPVLDSDGSFFLYSKLTVDKSRWQQGNVFSCSVMHEALHNHYTQKSLSLSPGK

SEQ ID NO: 17 - protein, 451 aa, synthetic construct
EVQLLESGGGLVQPGGSLRLSCAASGFTFNSYAMSWVRQAPGKGLEWVASIKSSGDRVQYADSVKGRFTISRDNSKNTVYLQMNSLRAEDTAIYYCAKPQWSSPQRTFEVWGQGTPVTVSSASTKGPSVFPLAPSSKSTSGGTAALGCLVKDYFPEPVTVSWNSGALTSGVHTFPAVLQSSGLYSLSSVVTVPSSSLGTQTYICNVNHKPSNTKVDKRVEPKSCDKTHTCPPCPAPELLGGPSVFLFPPKPKDTLMISRTPEVTCVVVDVSHEDPEVKFNWYVDGVEVHNAKTKPREEQYNSTYRVVSVLTVLHQDWLNGKEYKCKVSNKALPAPIEKTISKAKGQPREPQVYTLPPSRDELTKNQVSLTCLVKGFYPSDIAVEWESNGQPENNYKTTPPVLDSDGSFFLYSKLTVDKSRWQQGNVFSCSVMHEALHNHYTQKSLSLSPGK

SEQ ID NO: 18 - protein, 451 aa, synthetic construct
EVQLLESGGGLVQPGGSLRLSCAASGFTFNSYAMSWVRQAPGKGLEWVASIKSSGDRVQYADSVKGRFTISRDNSKNTVYLQMNSLRAEDTAIYYCAKPQWSSPQRTFEVWGQGTMVTVSSASTKGPSVFPLAPSSKSTSGGTAALGCLVKDYFPEPVTVSWNSGALTSGVHTFPAVLQSSGLYSLSSVVTVPSSSLGTQTYICNVNHKPSNTKVDKRVEPKSCDKTHTCPPCPAPELLGGPSVFLFPPKPKDTLMISRTPEVTCVVVDVSHEDPEVKFNWYVDGVEVHNAKTKPREEQYNSTYRVVSVLTVLHQDWLNGKEYKCKVSNKALPAPIEKTISKAKGQPREPQVYTLPPSRDELTKNQVSLTCLVKGFYPSDIAVEWESNGQPENNYKTTPPVLDSDGSFFLYSKLTVDKSRWQQGNVFSCSVMHEALHNHYTQKSLSLSPGK

SEQ ID NO: 19 - protein, 330 aa, synthetic construct
ASTKGPSVFPLAPSSKSTSGGTAALGCLVKDYFPEPVTVSWNSGALTSGVHTFPAVLQSSGLYSLSSVVTVPSSSLGTQTYICNVNHKPSNTKVDKRVEPKSCDKTHTCPPCPAPEAAGGPCVFLFPPKPKDTLMISRTPEVTCVVVDVSHEDPEVKFNWYVDGVEVHNAKTKPREEQYNSTYRVVSVLTVLHQDWLNGKEYKCKVSNKALGAPIEKTISKAKGQPREPQVYTLPPSRDELTKNQVSLTCLVKGFYPSDIAVEWESNGQPENNYKTTPPVLDSDGSFFLYSKLTVDKSRWQQGNVFSCSVMHEALHNHYTQKSLSLSPGK

SEQ ID NO: 20 - protein, 330 aa, synthetic construct
ASTKGPSVFPLAPSSKSTSGGTAALGCLVKDYFPEPVTVSWNSGALTSGVHTFPAVLQSSGLYSLSSVVTVPSSSLGTQTYICNVNHKPSNTKVDKRVEPKSCDKTHTCPPCPAPEAAGGPCVFLFPPKPKDTLMISRTPEVTCVVVDVSHEDPEVKFNWYVDGVEVHNAKTKPREEQYNSTYRVVSVLTVLHQDWLNGKEYKCKVSNKALGAPIEKTISKAKGQPREPQVYTLPPSRDELTKNQVSLTCLVKGFYPSDIAVEWESNGQPENNYKTTPPVLDSDGSFFLYSKLTVDKSRWQQGNVFSCSVLHEALHSHYTQKSLSLSPGK

SEQ ID NO: 21 - protein, 220 aa, synthetic construct
DIVMTQSPDSLAVSLGERATINCKSSQSLLYSSNQKNYLAWYQQKPGQPPKLLIYWASSRESGVPDRFSGSGSGTDFTLTISSLQAEDVAVYYCQQYYNYPLTFGQGTKLEIKRTVAAPSVFIFPPSDEQLKSGTASVVCLLNNFYPREAKVQWKVDNALQSGNSQESVTEQDSKDSTYSLSSTLTLSKADYEKHKVYACEVTHQGLSSPVTKSFNRGEC

SEQ ID NO: 22 - protein, 446 aa, synthetic construct
EVQLVESGGGLVQPGGSLRLSCAASGFTFNKNAMNWVRQAPGKGLEWVGRIRNKTNNYATYYADSVKGRFTISRDDSKNSLYLQMNSLKTEDTAVYYCVAGNSFAYWGQGTLVTVSASTKGPSVFPLAPSSKSTSGGTAALGCLVKDYFPEPVTVSWNSGALTSGVHTFPAVLQSSGLYSLSSVVTVPSSSLGTQTYICNVNHKPSNTKVDKRVEPKSCDKTHTCPPCPAPEAAGGPCVFLFPPKPKDTLMISRTPEVTCVVVDVSHEDPEVKFNWYVDGVEVHNAKTKPREEQYNSTYRVVSVLTVLHQDWLNGKEYKCKVSNKALGAPIEKTISKAKGQPREPQVYTLPPSRDELTKNQVSLTCLVKGFYPSDIAVEWESNGQPENNYKTTPPVLDSDGSFFLYSKLTVDKSRWQQGNVFSCSVLHEALHSHYTQKSLSLSPGK

SEQ ID NO: 23 - protein, 121 aa, synthetic construct
EVQLLESGGGLVQPGGSLRLSCAASGFTFNSYAMSWVRQAPGKGLEWVASIKSSGDRVQYADSVKGRFTISRDNSKNTVYLQMNSLRAEDTAIYYCAKPRWSSPQRTFEVWGQGTMVTVSS

SEQ ID NO: 24 - protein, 121 aa, synthetic construct
EVQLLESGGGLVQPGGSLRLSCAASGFTFNSYAMSWVRQAPGKGLEWVASIKSSGDRVQYADSVKGRFTISRDNSKNTVYLQMNSLRAEDTAIYYCAKPQWRSPQRTFEVWGQGTMVTVSS

SEQ ID NO: 25 - protein, 121 aa, synthetic construct
EVQLLESGGGLVQPGGSLRLSCAASGFTFNSYAMSWVRQAPGKGLEWVASIKSSGARVQYADSVKGRFTISRDNSKNTVYLQMNSLRAEDTAIYYCAKPQWSSPQRTFEVWGQGTMVTVSS

SEQ ID NO: 26 - protein, 121 aa, synthetic construct
EVQLLESGGGLVQPGGSLRLSCAASGFTFNSYAMSWVRQAPGKGLEWVASIKSSGKRVQYADSVKGRFTISRDNSKNTVYLQMNSLRAEDTAIYYCAKPRWSSPQRTFEVWGQGTMVTVSS

SEQ ID NO: 27 - protein, 121 aa, synthetic construct
EVQLLESGGGLVQPGGSLRLSCAASGFTFNSYAMSWVRQAPGKGLEWVASIKSSGARVQYADSVKGRFTISRDNSKNTVYLQMNSLRAEDTAIYYCAKPQWRSPQRTFEVWGQGTMVTVSS

SEQ ID NO: 28 - protein, 121 aa, synthetic construct
EVQLLESGGGLVQPGGSLRLSCAASGFTFNSYAMSWVRQAPGKGLEWVASIKSSGKRVQYADSVKGRFTISRDNSKNTVYLQMNSLRAEDTAIYYCAKPQWRSPQRTFEVWGQGTMVTVSS

SEQ ID NO: 29 - protein, 451 aa, synthetic construct
EVQLLESGGGLVQPGGSLRLSCAASGFTFNSYAMSWVRQAPGKGLEWVASIKSSGDRVQYADSVKGRFTISRDNSKNTVYLQMNSLRAEDTAIYYCAKPRWSSPQRTFEVWGQGTMVTVSSASTKGPSVFPLAPSSKSTSGGTAALGCLVKDYFPEPVTVSWNSGALTSGVHTFPAVLQSSGLYSLSSVVTVPSSSLGTQTYICNVNHKPSNTKVDKRVEPKSCDKTHTCPPCPAPEAAGGPCVFLFPPKPKDTLMISRTPEVTCVVVDVSHEDPEVKFNWYVDGVEVHNAKTKPREEQYNSTYRVVSVLTVLHQDWLNGKEYKCKVSNKALGAPIEKTISKAKGQPREPQVYTLPPSRDELTKNQVSLTCLVKGFYPSDIAVEWESNGQPENNYKTTPPVLDSDGSFFLYSKLTVDKSRWQQGNVFSCSVLHEALHSHYTQKSLSLSPGK

SEQ ID NO: 30 - protein, 451 aa, synthetic construct
EVQLLESGGGLVQPGGSLRLSCAASGFTFNSYAMSWVRQAPGKGLEWVASIKSSGDRVQYADSVKGRFTISRDNSKNTVYLQMNSLRAEDTAIYYCAKPQWRSPQRTFEVWGQGTMVTVSSASTKGPSVFPLAPSSKSTSGGTAALGCLVKDYFPEPVTVSWNSGALTSGVHTFPAVLQSSGLYSLSSVVTVPSSSLGTQTYICNVNHKPSNTKVDKRVEPKSCDKTHTCPPCPAPEAAGGPCVFLFPPKPKDTLMISRTPEVTCVVVDVSHEDPEVKFNWYVDGVEVHNAKTKPREEQYNSTYRVVSVLTVLHQDWLNGKEYKCKVSNKALGAPIEKTISKAKGQPREPQVYTLPPSRDELTKNQVSLTCLVKGFYPSDIAVEWESNGQPENNYKTTPPVLDSDGSFFLYSKLTVDKSRWQQGNVFSCSVLHEALHSHYTQKSLSLSPGK

SEQ ID NO: 31 - protein, 451 aa, synthetic construct
EVQLLESGGGLVQPGGSLRLSCAASGFTFNSYAMSWVRQAPGKGLEWVASIKSSGARVQYADSVKGRFTISRDNSKNTVYLQMNSLRAEDTAIYYCAKPQWSSPQRTFEVWGQGTMVTVSSASTKGPSVFPLAPSSKSTSGGTAALGCLVKDYFPEPVTVSWNSGALTSGVHTFPAVLQSSGLYSLSSVVTVPSSSLGTQTYICNVNHKPSNTKVDKRVEPKSCDKTHTCPPCPAPEAAGGPCVFLFPPKPKDTLMISRTPEVTCVVVDVSHEDPEVKFNWYVDGVEVHNAKTKPREEQYNSTYRVVSVLTVLHQDWLNGKEYKCKVSNKALGAPIEKTISKAKGQPREPQVYTLPPSRDELTKNQVSLTCLVKGFYPSDIAVEWESNGQPENNYKTTPPVLDSDGSFFLYSKLTVDKSRWQQGNVFSCSVLHEALHSHYTQKSLSLSPGK

SEQ ID NO: 32 - protein, 451 aa, synthetic construct
EVQLLESGGGLVQPGGSLRLSCAASGFTFNSYAMSWVRQAPGKGLEWVASIKSSGKRVQYADSVKGRFTISRDNSKNTVYLQMNSLRAEDTAIYYCAKPRWSSPQRTFEVWGQGTMVTVSSASTKGPSVFPLAPSSKSTSGGTAALGCLVKDYFPEPVTVSWNSGALTSGVHTFPAVLQSSGLYSLSSVVTVPSSSLGTQTYICNVNHKPSNTKVDKRVEPKSCDKTHTCPPCPAPEAAGGPCVFLFPPKPKDTLMISRTPEVTCVVVDVSHEDPEVKFNWYVDGVEVHNAKTKPREEQYNSTYRVVSVLTVLHQDWLNGKEYKCKVSNKALGAPIEKTISKAKGQPREPQVYTLPPSRDELTKNQVSLTCLVKGFYPSDIAVEWESNGQPENNYKTTPPVLDSDGSFFLYSKLTVDKSRWQQGNVFSCSVLHEALHSHYTQKSLSLSPGK

SEQ ID NO: 33 - protein, 451 aa, synthetic construct
EVQLLESGGGLVQPGGSLRLSCAASGFTFNSYAMSWVRQAPGKGLEWVASIKSSGARVQYADSVKGRFTISRDNSKNTVYLQMNSLRAEDTAIYYCAKPQWRSPQRTFEVWGQGTMVTVSSASTKGPSVFPLAPSSKSTSGGTAALGCLVKDYFPEPVTVSWNSGALTSGVHTFPAVLQSSGLYSLSSVVTVPSSSLGTQTYICNVNHKPSNTKVDKRVEPKSCDKTHTCPPCPAPEAAGGPCVFLFPPKPKDTLMISRTPEVTCVVVDVSHEDPEVKFNWYVDGVEVHNAKTKPREEQYNSTYRVVSVLTVLHQDWLNGKEYKCKVSNKALGAPIEKTISKAKGQPREPQVYTLPPSRDELTKNQVSLTCLVKGFYPSDIAVEWESNGQPENNYKTTPPVLDSDGSFFLYSKLTVDKSRWQQGNVFSCSVLHEALHSHYTQKSLSLSPGK

SEQ ID NO: 34 - protein, 451 aa, synthetic construct
EVQLLESGGGLVQPGGSLRLSCAASGFTFNSYAMSWVRQAPGKGLEWVASIKSSGKRVQYADSVKGRFTISRDNSKNTVYLQMNSLRAEDTAIYYCAKPQWRSPQRTFEVWGQGTMVTVSSASTKGPSVFPLAPSSKSTSGGTAALGCLVKDYFPEPVTVSWNSGALTSGVHTFPAVLQSSGLYSLSSVVTVPSSSLGTQTYICNVNHKPSNTKVDKRVEPKSCDKTHTCPPCPAPEAAGGPCVFLFPPKPKDTLMISRTPEVTCVVVDVSHEDPEVKFNWYVDGVEVHNAKTKPREEQYNSTYRVVSVLTVLHQDWLNGKEYKCKVSNKALGAPIEKTISKAKGQPREPQVYTLPPSRDELTKNQVSLTCLVKGFYPSDIAVEWESNGQPENNYKTTPPVLDSDGSFFLYSKLTVDKSRWQQGNVFSCSVLHEALHSHYTQKSLSLSPGK

SEQ ID NO: 35 - protein, 580 aa, synthetic construct
MAGTVRTACLVVAMLLSLDFPGQAQPPPPPPDATCHQVRSFFQRLQPGLKWVPETPVPGSDLQVCLPKGPTCCSRKMEEKYQLTARLNMEQLLQSASMELKFLIIQNAAVFQEAFEIVVRHAKNYTNAMFKNNYPSLTPQAFEFVGEFFTDVSLYILGSDINVDDMVNELFDSLFPVIYTQLMNPGLPDSALDINECLRGARRDLKVFGNFPKLIMTQVSKSLQVTRIFLQALNLGIEVINTTDHLKFSKDCGRMLTRMWYCSYCQGLMMVKPCGGYCNVVMQGCMAGVVEIDKYWREYILSLEELVNGMYRIYDMENVLLGLFSTIHDSIQYVQKNAGKLTTTIGKLCAHSQQRQYRSAYYPEDLFIDKKVLKVAHVEHEETLSSRRRELIQKLKSFISFYSALPGYICSHSPVAENDTLCWNGQELVERYSQKAARNGMKNQFNLHELKMKGPEPVVSQIIDKLKHINQLLRTMSMPKGRVLDKNLDEEGFESGDCGDDEDECIGGSGDGMIKVKNQLRFLAELAYDLDVDDAPGNSQQATPKDNEISTFHNLGNVHSPLKLLTSMAISVVCFFFLVH

SEQ ID NO: 36 - protein, 51 aa, synthetic construct
GDGMIKVKNQLRFLAELAYDLDVDDAPGNSQQATPKDNEISTFHNLGNVHS

SEQ ID NO: 37 - protein, 54 aa, synthetic construct
MPKGRVLDKNLDEEGFESGDCGDDEDECIGGSGDGMIKVKNQLRFLAELAYDLD

SEQ ID NO: 38 - protein, 12 aa, synthetic construct
DKNLDEEGFESG

SEQ ID NO: 39 - protein, 107 aa, synthetic construct
DIQLTQSPSSLSASVGDRVTITCQASQDIDNSVTWYQQRPGKAPSLLISDASILESGVPSRFSGRGSGTHFTLSITSLQPEDIATYYCQQYENLPITFGQGTRLEIK

SEQ ID NO: 40 - protein, 121 aa, synthetic construct
EVQLLESGGGLVQPGGSMRLSCAASEIDFSVYALGWSRQAPGKQRELVATITTSSTTTYADSVKGRFTISRDNAKNTVYLQMNSLKPEDTAVYYCHTLRRTGSGIVPGRIWGQGTPVTVSS

SEQ ID NO: 41 - protein, 107 aa, synthetic construct
DIQMIQSPSSLSASVGDRVTITCRASQSISSYLNWYQQKPGKAPKLLIYAASSLQSGVPSRFSGSGSGTDFTLTISSLQPEDFATYYCQQGYSTPFTLGPGTKVDIK

SEQ ID NO: 42 - protein, 118 aa, synthetic construct
EVQLLESGGGVVQPGRSLRLSCAASGFTFSSYAMHWVRQAPGKGLEWVAVISYDGSNKYYADSVKGRFTISRDNSKNTLYLQMNSLRAEDTAVYYCARDESRRKFDYWGQGTTVTVSS

SEQ ID NO: 43 - protein, 107 aa, synthetic construct
NIQMTQSPSSLSASVGDRVTITCRASQSITRYLNWYQQKPGKGPKLLIYAASRLQSGVPSRFSGSGSGTDFTLTISSLQPEDFATYYCQQSHSIPRTFGQGTKLEIK

SEQ ID NO: 44 - protein, 115 aa, synthetic construct
EVQLLESGGGVVQPGRSLRLSCAASGFTFSSYGMHWVRQAPGKGLEWVAVISYDGSNKYYADSVKGRFTISRDNSKNTLYLQMNSLRAEDTAVYYCAKNPSLDYWGQGTTVTVSS

SEQ ID NO: 45 - protein, 107 aa, synthetic construct
DIQLTQSPSSLSASVGDRVTITCRASQSISSYLSWYQQKPGKAPKLLIYGASSLQSGVPSRFSGSGSGTDFTLTISSLQPEDFATYSCQQSYSTQFTFGPGTKVDIK

SEQ ID NO: 46 - protein, 117 aa, synthetic construct
EVQLLESGGGVVQPGRSLRLSCAASGFTFSSYAMHWVRQAPGKGLEWVAVISYDGSNKYYADSVKGRFTISRDNSKNTLYLQMNSLRAEDTAVYYCARRQRAAIDYWGQGTTVTVSS

SEQ ID NO: 47 - protein, 107 aa, synthetic construct
DIQLTQSPSSLSASVGDRVTITCRAGQTINNYLHWYQQKPGKAPKLLIFAASSLQSGVPSRFSGSGSGTDFTLTISSLQPEDFATYYCQQSYSPPLTFGGGTRVEIK

SEQ ID NO: 48 - protein, 118 aa, synthetic construct
EVQLLESGGGVVRPGRSLRLSCAASGFTFSSYAMHWVRQAPGKGLEWVAVISYDGSNKYYADSVKGRFTISRDNSKNTLYLQMNSLRAEDTAVYYCARRKSGSSFDYWGQGTPVTVSS

SEQ ID NO: 49 - protein, 107 aa, synthetic construct
AIRLTQFPSSLSASVGDRVTITCRARQSIDNYLNWYQEKPGKAPKLLIYAASSLQSGVPSRFSGSGSGTEFTLTISSLQPDDFAAYYCQQSYDSPPTFGQGTKVEIK

SEQ ID NO: 50 - protein, 121 aa, synthetic construct
EVQLLESGGGLVQPGGSLRLSCAASGFTFSSYAMHWVRQAPGKGLEYVSAISSNGGSTYYANSVKGRFTISRHPSKNILFLEMNSLRPDDTAVYYCVRGWIRPPPGSFDLWGQGTPVTVSS

SEQ ID NO: 51 - protein, 107 aa, synthetic construct
NIQMTQSPSSLSAFVGDRVTITCRASQSISRYLNWYQHKPGQAPKLLMYAASTLQDEVPSRFSGSGSGTYFTLTISSLEPEDFATYYCQQSYSTPPTFGGGTKVEIK

SEQ ID NO: 52 - protein, 121 aa, synthetic construct
EVQLLESGGGLVQPGGSLRLSCAASGFTFSSYAMHWVRQAPGKGLEYVSAISSNGGSTYYANSVKGRFTISRDNSKNTLYLQMGSLRPDDTAVYYCVRGWIRPPPGSFDLWGQGTTVTVSS

SEQ ID NO: 53 - protein, 107 aa, synthetic construct
NIQMTQSPSSLSASVGDRVTITCRASQSISSYLNWYQQKPGKAPKLLIYAASSLQSGVPSRFSGSGSGTDFTLTISSLQPEDFATYYCQQSYSTPLTFGGGTKVEIK

SEQ ID NO: 54 - protein, 118 aa, synthetic construct
EVQLLESGGGVVQPGRSLRLSCAASGFTFSSYAMHWVRQAPGKGLEWVAVISYDGSNKYYADSVKGRFTISRDNSKNTLYLQMNSLRAEDTAVYYCARRLRGSGMDVWGQGTPVTVSS

SEQ ID NO: 55 - protein, 107 aa, synthetic construct
DIQLTQSPSSLSASVGDRVTITCRASQSISSYLNWYQQKPGKAPKLLIYAASSLQSGVPSRFSGSGSGTDFTLTISSLQPEDFATYYCQQSYSTPPTFGPGTKVDIK

SEQ ID NO: 56 - protein, 121 aa, synthetic construct
EVQLVESGGGLIQPGGSLRLSCAASGFTFSSYAMHWVRQAPGKGLEYVSAISSNGGSTYYADSVKGRFTISRDNSKNTLYLQMSSLRPDDTAVYYCVRGWIRPPPGSFDLWGQGTTVTVSS

SEQ ID NO: 57 - protein, 107 aa, synthetic construct
AIRLTQSPSSLSASVGDRVSITCRASQSISTFLNWYQQKPGKAPNLLIYSASTLQSGVPSRFSGSGSGTDFTLTISSLQPEDFATYYCQQSYSSPPTFGQGTKLEIK

SEQ ID NO: 58 - protein, 121 aa, synthetic construct
EVQLVESGGGLVQPGGSLRLSCAASGFTFSSYAMHWVRQAPGKGLEYVSAISSNGGSTYYANSVKGRFTISRDNSKNTLYLQMGSLRAEDMAVYYCVRGWIRPPPGSFDLWGQGTPVTVSS